European Patent Application EP 4 659 811 A1, published December 10, 2025. Title: BK VIRUS NEUTRALIZING ANTIBODIES. Applicant: UNIVERSITE DE STRASBOURG. The sequence listing filed with the application follows.

SEQUENCE LISTING (274 sequences)

SEQ ID NO: 1 - protein, 8 aa, synthetic construct
  VARIANT 8: note = X is T or S
GFTFRSYX

SEQ ID NO: 2 - protein, 8 aa, synthetic construct
  VARIANT 7: note = X is H or Q
ISGSSNXK

SEQ ID NO: 3 - protein, 15 aa, Homo sapiens
AREDDILTPLYGMDV

SEQ ID NO: 4 - protein, 7 aa, Homo sapiens
QSVRSNY

SEQ ID NO: 5 - protein, 9 aa, synthetic construct
  VARIANT 4: note = X is G or A
HQYXSSPRT

SEQ ID NO: 6 - protein, 8 aa, Homo sapiens
GFTFRSYT

SEQ ID NO: 7 - protein, 8 aa, Homo sapiens
ISGSSNHK

SEQ ID NO: 8 - protein, 9 aa, Homo sapiens
HQYGSSPRT

SEQ ID NO: 9 - protein, 8 aa, Homo sapiens
GFTFRSYS

SEQ ID NO: 10 - protein, 8 aa, Homo sapiens
ISGSSNQK

SEQ ID NO: 11 - protein, 9 aa, Homo sapiens
HQYASSPRT

SEQ ID NO: 12 - protein, 8 aa, Homo sapiens
AYTFTNSA

SEQ ID NO: 13 - protein, 8 aa, Homo sapiens
INTNTGNP

SEQ ID NO: 14 - protein, 20 aa, synthetic construct
  VARIANT 1: note = X is T or A
  VARIANT 13: note = X is Y or F
  VARIANT 14: note = X is Y or H
  VARIANT 18: note = X is V or M
  VARIANT 20: note = X is I or V
XVPYNFGGDHNSXXFFGXDX

SEQ ID NO: 15 - protein, 9 aa, synthetic construct
  VARIANT 6: note = X is S or T
  VARIANT 9: note = X is L or F
SSDVGXYNX

SEQ ID NO: 16 - protein, 10 aa, synthetic construct
  VARIANT 1: note = X is C or S
  VARIANT 6: note = X is S or G
  VARIANT 8: note = X is T or A
XSYAGXNXFV

SEQ ID NO: 17 - protein, 20 aa, Homo sapiens
TVPYNFGGDHNSYYFFGVDI

SEQ ID NO: 18 - protein, 9 aa, Homo sapiens
SSDVGSYNL

SEQ ID NO: 19 - protein, 10 aa, Homo sapiens
CSYAGSNTFV

SEQ ID NO: 20 - protein, 20 aa, Homo sapiens
AVPYNFGGDHNSFHFFGMDV

SEQ ID NO: 21 - protein, 9 aa, Homo sapiens
SSDVGTYNF

SEQ ID NO: 22 - protein, 10 aa, Homo sapiens
SSYAGGNAFV

SEQ ID NO: 23 - protein, 8 aa, Homo sapiens
GGSIRNSY

SEQ ID NO: 24 - protein, 7 aa, synthetic construct
  VARIANT 6: note = X is T or S
IYYTGXT

SEQ ID NO: 25 - protein, 11 aa, Homo sapiens
AQGGGSGDLHY

SEQ ID NO: 26 - protein, 9 aa, Homo sapiens
RSDVGGYNY

SEQ ID NO: 27 - protein, 10 aa, Homo sapiens
ISFATGYTWV

SEQ ID NO: 28 - protein, 7 aa, Homo sapiens
IYYTGTT

SEQ ID NO: 29 - protein, 7 aa, Homo sapiens
IYYTGST

SEQ ID NO: 30 - protein, 8 aa, Homo sapiens
GGSISPYY

SEQ ID NO: 31 - protein, 7 aa, Homo sapiens
IYYSGNT

SEQ ID NO: 32 - protein, 18 aa, synthetic construct
  VARIANT 13: note = X is D or G
ARDSCSGTCYLGXNWFDP

SEQ ID NO: 33 - protein, 9 aa, Homo sapiens
SSNIGANND

SEQ ID NO: 34 - protein, 12 aa, Homo sapiens
QSYDSSLSTSKV

SEQ ID NO: 35 - protein, 18 aa, Homo sapiens
ARDSCSGTCYLGDNWFDP

SEQ ID NO: 36 - protein, 18 aa, Homo sapiens
ARDSCSGTCYLGGNWFDP

SEQ ID NO: 37 - protein, 8 aa, Homo sapiens
GFTFESYG

SEQ ID NO: 38 - protein, 8 aa, Homo sapiens
ISNDGSIE

SEQ ID NO: 39 - protein, 20 aa, Homo sapiens
AKDAVGITGGSLYYSYGMDV

SEQ ID NO: 40 - protein, 6 aa, Homo sapiens
QTIKNY

SEQ ID NO: 41 - protein, 9 aa, Homo sapiens
QQSYSAPYS

SEQ ID NO: 42 - protein, 8 aa, Homo sapiens
GFTVSTNC

SEQ ID NO: 43 - protein, 7 aa, Homo sapiens
IYSGGTT

SEQ ID NO: 44 - protein, 14 aa, Homo sapiens
ARSVDTYDIYALDV

SEQ ID NO: 45 - protein, 6 aa, Homo sapiens
QSISRW

SEQ ID NO: 46 - protein, 9 aa, Homo sapiens
QQYNSYPWT

SEQ ID NO: 47 - protein, 8 aa, Homo sapiens
GFTFDDHA

SEQ ID NO: 48 - protein, 8 aa, Homo sapiens
INWNSASI

SEQ ID NO: 49 - protein, 16 aa, Homo sapiens
AKDFGLWFGESRGIDA

SEQ ID NO: 50 - protein, 11 aa, Homo sapiens
QSLLHSNGYNY

SEQ ID NO: 51 - protein, 9 aa, Homo sapiens
MQALQTPIT

SEQ ID NO: 52 - protein, 10 aa, Homo sapiens
GGSISSGGYY

SEQ ID NO: 53 - protein, 7 aa, Homo sapiens
MYYSGST

SEQ ID NO: 54 - protein, 17 aa, Homo sapiens
ARDRRDYGDYYYFGMDV

SEQ ID NO: 55 - protein, 9 aa, Homo sapiens
SSNIGAGYD

SEQ ID NO: 56 - protein, 12 aa, Homo sapiens
QSYDSSLSVYVV

SEQ ID NO: 57 - protein, 8 aa, Homo sapiens
GFTFTNYW

SEQ ID NO: 58 - protein, 8 aa, Homo sapiens
IYPDDSDA

SEQ ID NO: 59 - protein, 19 aa, Homo sapiens
ARGGFCSGSVCYNPAWFDL

SEQ ID NO: 60 - protein, 6 aa, Homo sapiens
QTINTY

SEQ ID NO: 61 - protein, 9 aa, Homo sapiens
QQSYSTPLT

SEQ ID NO: 62 - protein, 8 aa, Homo sapiens
GYTFTTHI

SEQ ID NO: 63 - protein, 8 aa, Homo sapiens
INAGNGNT

SEQ ID NO: 64 - protein, 14 aa, Homo sapiens
AREDQWLGRSPLEY

SEQ ID NO: 65 - protein, 7 aa, Homo sapiens
QSVSSSY

SEQ ID NO: 66 - protein, 10 aa, Homo sapiens
QQYGNSYPWT

SEQ ID NO: 67 - protein, 8 aa, synthetic construct
  VARIANT 3: note = X is T or P
GFXFSSYA

SEQ ID NO: 68 - protein, 8 aa, synthetic construct
  VARIANT 1: note = X is L or I
  VARIANT 5: note = X is G or A
  VARIANT 6: note = X is G or S
  VARIANT 7: note = X is S or G
XTGSXXXT

SEQ ID NO: 69 - protein, 15 aa, synthetic construct
  VARIANT 10: note = X is F or Y
AKEGAYSYDXWYFDL

SEQ ID NO: 70 - protein, 7 aa, synthetic construct
  VARIANT 2: note = X is T or S
  VARIANT 6: note = X is N or S
QXVSGXY

SEQ ID NO: 71 - protein, 8 aa, synthetic construct
  VARIANT 5: note = X is R or S
  VARIANT 6: note = X is P or L
  VARIANT 7: note = X is L or V
QQYGXXXT

SEQ ID NO: 72 - protein, 8 aa, Homo sapiens
GFTFSSYA

SEQ ID NO: 73 - protein, 8 aa, Homo sapiens
LTGSGGST

SEQ ID NO: 74 - protein, 15 aa, Homo sapiens
AKEGAYSYDFWYFDL

SEQ ID NO: 75 - protein, 7 aa, Homo sapiens
QTVSGNY

SEQ ID NO: 76 - protein, 8 aa, Homo sapiens
QQYGRPLT

SEQ ID NO: 77 - protein, 8 aa, Homo sapiens
GFPFSSYA

SEQ ID NO: 78 - protein, 8 aa, Homo sapiens
ITGSASGT

SEQ ID NO: 79 - protein, 15 aa, Homo sapiens
AKEGAYSYDYWYFDL

SEQ ID NO: 80 - protein, 7 aa, Homo sapiens
QSVSGSY

SEQ ID NO: 81 - protein, 8 aa, Homo sapiens
QQYGSLVT

SEQ ID NO: 82 - protein, 8 aa, Homo sapiens
GFTFSNFG

SEQ ID NO: 83 - protein, 8 aa, Homo sapiens
ISYDGSDK

SEQ ID NO: 84 - protein, 19 aa, Homo sapiens
AKDRVRTKYYYDHSGPFDY

SEQ ID NO: 85 - protein, 6 aa, Homo sapiens
NIGSKS

SEQ ID NO: 86 - protein, 11 aa, Homo sapiens
QVWMTNSDRPV

SEQ ID NO: 87 - protein, 8 aa, Homo sapiens
GFTFSSYG

SEQ ID NO: 88 - protein, 8 aa, Homo sapiens
ISKDGSNK

SEQ ID NO: 89 - protein, 19 aa, Homo sapiens
AKIPLRRYSDSGDYSSGDF

SEQ ID NO: 90 - protein, 11 aa, Homo sapiens
ENLVYSDGNTY

SEQ ID NO: 91 - protein, 10 aa, Homo sapiens
MQTTHWPPLT

SEQ ID NO: 92 - protein, 8 aa, Homo sapiens
GFIFNNHG

SEQ ID NO: 93 - protein, 8 aa, Homo sapiens
ISYDGKKE

SEQ ID NO: 94 - protein, 13 aa, Homo sapiens
AKEAYGSGSPCDY

SEQ ID NO: 95 - protein, 7 aa, Homo sapiens
QRVSSNY

SEQ ID NO: 96 - protein, 9 aa, Homo sapiens
QQYGTSPRS

SEQ ID NO: 97 - protein, 8 aa, synthetic construct
  VARIANT 3: note = X is S or R
  VARIANT 6: note = X is S or T
GFXFGXYS

SEQ ID NO: 98 - protein, 8 aa, Homo sapiens
ISSGSSSI

SEQ ID NO: 99 - protein, 12 aa, Homo sapiens
ARGWTGYDAFDI

SEQ ID NO: 100 - protein, 6 aa, Homo sapiens
QVISNY

SEQ ID NO: 101 - protein, 9 aa, Homo sapiens
QKYNNAPLT

SEQ ID NO: 102 - protein, 8 aa, Homo sapiens
GFSFGSYS

SEQ ID NO: 103 - protein, 8 aa, Homo sapiens
GFRFGTYS

SEQ ID NO: 104 - protein, 8 aa, synthetic construct
  VARIANT 4: note = X is L or S
  VARIANT 6: note = X is N or G
GFSXSXSE

SEQ ID NO: 105 - protein, 10 aa, synthetic construct
  VARIANT 4: note = X is R or T
  VARIANT 10: note = X is T or P
VRSXANRHAX

SEQ ID NO: 106 - protein, 15 aa, synthetic construct
TGVRGVISRYFAMDV

SEQ ID NO: 107 - protein, 9 aa, synthetic construct
  VARIANT 1: note = X is S or N
  VARIANT 4: note = X is V or L
  VARIANT 6: note = X is A or S
XSDXGXYNY

SEQ ID NO: 108 - protein, 10 aa, synthetic construct
  VARIANT 5: note = X is H or S
  VARIANT 6: note = X is R or V
  VARIANT 8: note = X is T or S
  VARIANT 10: note = X is L or I
CSYAXXGXPX

SEQ ID NO: 109 - protein, 8 aa, Homo sapiens
GFSLSNSE

SEQ ID NO: 110 - protein, 10 aa, Homo sapiens
VRSRANRHAT

SEQ ID NO: 111 - protein, 9 aa, Homo sapiens
SSDVGAYNY

SEQ ID NO: 112 - protein, 10 aa, Homo sapiens
CSYAHRGTPL

SEQ ID NO: 113 - protein, 8 aa, Homo sapiens
GFSSSGSE

SEQ ID NO: 114 - protein, 10 aa, Homo sapiens
VRSTANRHAP

SEQ ID NO: 115 - protein, 9 aa, Homo sapiens
SSDLGSYNY

SEQ ID NO: 116 - protein, 10 aa, Homo sapiens
CSYASVGSPI

SEQ ID NO: 117 - protein, 8 aa, Homo sapiens
GFTFSGSE

SEQ ID NO: 118 - protein, 6 aa, Homo sapiens
NIGSNS

SEQ ID NO: 119 - protein, 11 aa, Homo sapiens
QVWDRRGDLLV

SEQ ID NO: 120 - protein, 10 aa, synthetic construct
  VARIANT 2: note = X is G or T
  VARIANT 7: note = X is S or N
GXYISTXSYY

SEQ ID NO: 121 - protein, 7 aa, synthetic construct
  VARIANT 4: note = X is S or G
IEYXGST

SEQ ID NO: 122 - protein, 21 aa, synthetic construct
  VARIANT 6: note = X is K or H
  VARIANT 14: note = X is Y or C
  VARIANT 17: note = X is G or S
  VARIANT 21: note = X is L or I
ASANSXYYDSGGYXAPXALDX

SEQ ID NO: 123 - protein, 6 aa, synthetic construct
  VARIANT 3: note = X is V or A
QSXSSH

SEQ ID NO: 124 - protein, 11 aa, synthetic construct
  VARIANT 10: note = X is Y or T
  VARIANT 11: note = X is S or absent
QQYNNWPPGXX

SEQ ID NO: 125 - protein, 10 aa, Homo sapiens
GGYISTSSYY

SEQ ID NO: 126 - protein, 7 aa, Homo sapiens
IEYSGST

SEQ ID NO: 127 - protein, 21 aa, Homo sapiens
ASANSKYYDSGGYYAPGALDL

SEQ ID NO: 128 - protein, 6 aa, Homo sapiens
QSVSSH

SEQ ID NO: 129 - protein, 11 aa, Homo sapiens
QQYNNWPPGYS

SEQ ID NO: 130 - protein, 10 aa, Homo sapiens
GTYISTNSYY

SEQ ID NO: 131 - protein, 7 aa, Homo sapiens
IEYGGST

SEQ ID NO: 132 - protein, 21 aa, Homo sapiens
ASANSHYYDSGGYCAPSALDI

SEQ ID NO: 133 - protein, 6 aa, Homo sapiens
QSASSH

SEQ ID NO: 134 - protein, 10 aa, Homo sapiens
QQYNNWPPGT

SEQ ID NO: 135 - protein, 10 aa, Homo sapiens
GGSISSGNYY

SEQ ID NO: 136 - protein, 7 aa, Homo sapiens
IYTSGNT

SEQ ID NO: 137 - protein, 13 aa, Homo sapiens
ARVRRDGYNAFDY

SEQ ID NO: 138 - protein, 6 aa, Homo sapiens
NLGDKF

SEQ ID NO: 139 - protein, 10 aa, Homo sapiens
QAWDSDTLYV

SEQ ID NO: 140 - protein, 10 aa, Homo sapiens
GGSMTSGSYY

SEQ ID NO: 141 - protein, 7 aa, Homo sapiens
IYTSGRT

SEQ ID NO: 142 - protein, 15 aa, Homo sapiens
ARWGDSSAYYYVGDP

SEQ ID NO: 143 - protein, 6 aa, Homo sapiens
QNINTY

SEQ ID NO: 144 - protein, 9 aa, Homo sapiens
QQSFSLPHT

SEQ ID NO: 145 - protein, 8 aa, Homo sapiens
GETYVGHS

SEQ ID NO: 146 - protein, 8 aa, Homo sapiens
ISLHNGNV

SEQ ID NO: 147 - protein, 23 aa, Homo sapiens
ARVPMKIYGVIVFGEYYYDQLDV

SEQ ID NO: 148 - protein, 9 aa, Homo sapiens
GSDVGGYNY

SEQ ID NO: 149 - protein, 9 aa, Homo sapiens
SSYAGSKVV

SEQ ID NO: 150 - protein, 8 aa, Homo sapiens
GYTFTSYS

SEQ ID NO: 151 - protein, 8 aa, Homo sapiens
INAGNGDT

SEQ ID NO: 152 - protein, 19 aa, Homo sapiens
ARSNSPTVTYNYYYYAMDV

SEQ ID NO: 153 - protein, 7 aa, Homo sapiens
QSVRSSY

SEQ ID NO: 154 - protein, 9 aa, Homo sapiens
QQYGNSPLT

SEQ ID NO: 155 - protein, 8 aa, Homo sapiens
GGRFSRYG

SEQ ID NO: 156 - protein, 8 aa, Homo sapiens
IIPLLGTA

SEQ ID NO: 157 - protein, 17 aa, Homo sapiens
ATARREYDRPGAEYFIQ

SEQ ID NO: 158 - protein, 6 aa, Homo sapiens
QSVSTN

SEQ ID NO: 159 - protein, 10 aa, Homo sapiens
QQYNYWPPLT

SEQ ID NO: 160 - protein, 8 aa, Homo sapiens
GFTFRSYA

SEQ ID NO: 161 - protein, 8 aa, Homo sapiens
LSSSGTTT

SEQ ID NO: 162 - protein, 16 aa, Homo sapiens
AKDRNAQWLGSEPLDP

SEQ ID NO: 163 - protein, 9 aa, Homo sapiens
QQAYTFPWT

SEQ ID NO: 164 - protein, 8 aa, Homo sapiens
GFTFSSYS

SEQ ID NO: 165 - protein, 8 aa, Homo sapiens
ISSSSRTI

SEQ ID NO: 166 - protein, 10 aa, Homo sapiens
ARQAVAHFDY

SEQ ID NO: 167 - protein, 8 aa, Homo sapiens
GFTFSTYT

SEQ ID NO: 168 - protein, 8 aa, Homo sapiens
ISSRSTSI

SEQ ID NO: 169 - protein, 14 aa, Homo sapiens
VRDRGYYGSNWFDS

SEQ ID NO: 170 - protein, 9 aa, Homo sapiens
SSDVGNYNY

SEQ ID NO: 171 - protein, 10 aa, Homo sapiens
CAYAGSYTLV

SEQ ID NO: 172 - protein, 10 aa, Homo sapiens
GGSISSGRYY

SEQ ID NO: 173 - protein, 7 aa, Homo sapiens
VYFSGST

SEQ ID NO: 174 - protein, 15 aa, Homo sapiens
ARAVRDYGDSYSFDY

SEQ ID NO: 175 - protein, 9 aa, Homo sapiens
SSDIGGYNY

SEQ ID NO: 176 - protein, 10 aa, Homo sapiens
CSYSIRGTPV

SEQ ID NO: 177 - protein, 122 aa, Homo sapiens
EVQLVESGGGLVQPGGSLRLSCAASGFTFRSYTMDWVRQAPGKGLEWVSCISGSSNHKYYADSVRGRFTISRDNAKNSLFLQMNSLRAEDSAVYYCAREDDILTPLYGMDVWGPGTTVTVSS

SEQ ID NO: 178 - protein, 108 aa, Homo sapiens
EIVLTQSPDTLSLSPGARATLSCRASQSVRSNYLAWYQQKPGQAPRLLIYGASSRATAIPDRFSGSGSGTDFTLTITRLEPEDFAVYYCHQYGSSPRTFGQGTKVEIK

SEQ ID NO: 179 - protein, 122 aa, Homo sapiens
EVQLVESGGGLVQPGGSLRLSCTASGFTFRSYTMDWVRQAPGKGLEWVSCISGSSNHKYYADSVRGRFTISRDNAKNSLLLQMNSLRAEDSAVYYCAREDDILTPLYGMDVWGPGTTVTVSS

SEQ ID NO: 180 - protein, 108 aa, Homo sapiens; identical to SEQ ID NO: 178

SEQ ID NO: 181 - protein, 122 aa, Homo sapiens
EVQLVESGGGLVQPGGSLRLSCAASGFTFRSYSMDWVRQAPGKGLEWVSYISGSSNQKYYTDSVRGRFTISRDNAKNSLFLQMNSLRAEDSAVYYCAREDDILTPLYGMDVWGPGTTVTVSS

SEQ ID NO: 182 - protein, 108 aa, Homo sapiens
EIVLTQSPDTLSLSPGARATLSCRASQSVRSNYLAWYQQKPGQAPRLLIYGASSRATAIPDRFSGSGSGTDFTLTITRLEPEDFAVYYCHQYASSPRTFGQGTKVEIK

SEQ ID NO: 183 - protein, 122 aa, Homo sapiens; identical to SEQ ID NO: 181

SEQ ID NO: 184 - protein, 108 aa, Homo sapiens
EIVLTQSPDTLSLSPGARATLSCRASQSVRSNYLAWYQQKPGQAPRLLIYGASSRATAIPDRFSGSGSGTDLTLTITRLEPEDFAVYYCHQYASSPRTFGQGTKVEIK

SEQ ID NO: 185 - protein, 127 aa, Homo sapiens
QVQLVQSGSELKKPGASVKVSCKASAYTFTNSAINWVRQAPGQGLEWMGWINTNTGNPAYAQGFRGRFVFSLDTSVSEAYLQISNLKAEDTATYYCTVPYNFGGDHNSYYFFGVDIWGQGTTVTVSS

SEQ ID NO: 186 - protein, 110 aa, Homo sapiens
QSALTQPASVSGSPGQSITISCTGSSSDVGSYNLVSWFQQHPAKAPKVMIYEGTKRPSGVSDRFSGSKSGNTASLTISGLQAEDEADYYCCSYAGSNTFVFGTGTKVSVL

SEQ ID NO: 187 - protein, 127 aa, Homo sapiens
QVQLVQSGSELKKPGASVRVSCKASAYTFTNSAINWVRQAPGQGLEWTGWINTNTGNPAYAQGFRGRFVFSLDTSVSEAYLQITNLKAEDTATYYCAVPYNFGGDHNSFHFFGMDVWGQGTTVTVSS

SEQ ID NO: 188 - protein, 110 aa, Homo sapiens
QSALTQPASVSGSPGQSITISCTGSSSDVGTYNFVSWYQQQPAKAPKVMIYEGTKRPSGISDRFSGSKSGNTASLTISGLQAEDEADYYCSSYAGGNAFVFGTGTRVSVL

SEQ ID NO: 189 - protein, 117 aa, Homo sapiens
QVQLQESGPGLVKPSETLSLTCTVSGGSIRNSYWSWIRQPPGKGLEWIGYIYYTGTTNSNPSLKSRATISVHMSQNQISLKLNSVTPADTAVYYCAQGGGSGDLHYWGQGTLVTVSS

SEQ ID NO: 190 - protein, 110 aa, Homo sapiens
NFMLTQPASVSGSPGQSITISCTGTRSDVGGYNYVSWYQQHPGKAPKLMIYDISSRPSGVSNRFSASKSGNTASLTISGLQAEDEADYYCISFATGYTWVFGGGTRLTVL

SEQ ID NO: 191 - protein, 117 aa, Homo sapiens
QVQLQESGPGLVKPSGTLSLTCTVSGGSIRNSYWSWIRQPPGKGLEWIGYIYYTGTTNSNPSLKSRVTISVHMSRNQISLKLNSVTPADTAVYYCAQGGGSGDLHYWGQGTLVTVSS

SEQ ID NO: 192 - protein, 110 aa, Homo sapiens; identical to SEQ ID NO: 190

SEQ ID NO: 193 - protein, 117 aa, Homo sapiens
QVQLQESGPGLVKPSETLSLTCTVSGGSIRNSYWSWIRQSPGKGLEWIGYIYYTGSTNSNPSLKSRLTVSVHMSQNQISLKLNSVTPADTAVYYCAQGGGSGDLHYWGQGTLVTVSS

SEQ ID NO: 194 - protein, 110 aa, Homo sapiens
QSALTQPASVSGSPGQSITISCTGTRSDVGGYNYVSWYQQHPGKAPKLIIYDISSRPSGVSNRFSASKSGNTASLTISGLQAEDEADYYCISFATGYTWVFGGGTSLTVL

SEQ ID NO: 195 - protein, 117 aa, Homo sapiens
QVQLQESGPGLVKPSETLSLTCTVSGGSIRNSYWSWIRQPPGKGLEWIGYIYYTGTTNSNPSLKSRVTISVHMSQNQISLKLNSVTPADTAVYYCAQGGGSGDLHYWGQGTLVTVSS

SEQ ID NO: 196 - protein, 108 aa, Homo sapiens; identical to SEQ ID NO: 182

SEQ ID NO: 197 - protein, 124 aa, Homo sapiens
QVQLQESGPGLVRPSETLSLTCTVSGGSISPYYWNWIRQPPGKGLEWIGYIYYSGNTKYNPSLKSRVTISVDTSKNQFSLKLSSVSAADTAVYYCARDSCSGTCYLGDNWFDPWGQGTLVTVSS

SEQ ID NO: 198 - protein, 112 aa, Homo sapiens
QSVLTQPPSVSGAPGQRVTISCTGSSSNIGANNDVHWYQHLPGTAPKLLIYGNNHRPSGVPDRFSGSKSGTSASLAITGLQAEDEADYYCQSYDSSLSTSKVFGGGTKLTVL

SEQ ID NO: 199 - protein, 124 aa, Homo sapiens; identical to SEQ ID NO: 197

SEQ ID NO: 200 - protein, 112 aa, Homo sapiens
QSVLTQPPPVSGAPGQRVTISCTGSSSNIGANNDVHWYQHLPGTAPKLLIYGNNHRPSGVPDRFSGSKSGTSASLAITGLQAEDEADYYCQSYDSSLSTSKVFGGGTKLTVL

SEQ ID NO: 201 - protein, 124 aa, Homo sapiens
QVQLQESGPGLVRPSETLSLTCTVSGGSISPYYWNWIRQPPGKGLEWIGYIYYSGNTKYNPSLKSRVTISVDTSKNQFSLKLSSVSAADTAVYYCARDSCSGTCYLGGNWFDPWGQGTLVTVSS

SEQ ID NO: 202 - protein, 112 aa, Homo sapiens; identical to SEQ ID NO: 198

SEQ ID NO: 203 - protein, 127 aa, Homo sapiens
EVQLVESGGGVVQPGRSLRLSCVTSGFTFESYGIHWVRQAPGKGLEWVAVISNDGSIEDYAGSVKGRFTISGDKAKNTVYLQVNSLRPDDTAVYYCAKDAVGITGGSLYYSYGMDVWGQGTTVTVSS

SEQ ID NO: 204 - protein, 107 aa, Homo sapiens
DIQMTQSPSPLSAFIGGRVTITCRASQTIKNYLNWYQQKPGEAPKLLIYTASTLQNGVPSRFSGSRSGTDFTLTITSLQPEDFATYYCQQSYSAPYSFGQGTKLEIK

SEQ ID NO: 205 - protein, 120 aa, Homo sapiens
EVQLVESGGGLIQPGGSLRLSCAASGFTVSTNCMSWVRQAPGTGLEWVSVIYSGGTTYYADSVKGRFTISRDNSRNTLYLQMNGLRAEDTAVYYCARSVDTYDIYALDVWGQGTTVTVSS

SEQ ID NO: 206 - protein, 107 aa, Homo sapiens
DIQMTQSPSTLSASVGDRVTITCRASQSISRWLAWYQQKPGKAPKLLIYKASGLHSGAPSRFSGSGSGTEFTLTISGLQPDDFATYFCQQYNSYPWTFGQGTKVEIK

SEQ ID NO: 207 - protein, 123 aa, Homo sapiens
EVQLVESGGGLVQPGRSLRLSCSASGFTFDDHAMHWVRQAPGKGLEWVAGINWNSASIVYADSVKGRFTISRDNVKNSLYLQMNSLRADDTALYYCAKDFGLWFGESRGIDAWGRGTTVTVSS

SEQ ID NO: 208 - protein, 112 aa, Homo sapiens
DIVMTQSPLSLPVTPGEPASISCRPSQSLLHSNGYNYLNWYLQKPGRSPQLLIYLGSNRASGVPDRFSGSGSGTDFTLKISRVEAEDVGIYYCMQALQTPITFGQGTRLEIK

SEQ ID NO: 209 - protein, 125 aa, Homo sapiens
QVQLQESGPGLVKPSQTLSLTCTVSGGSISSGGYYWSWIRQHPGKGLEWIGYMYYSGSTNYNPSLKSRVTISVDTSKNQFSLKLTSVTAADTAVYYCARDRRDYGDYYYFGMDVWGQGTTVTVSS

SEQ ID NO: 210 - protein, 112 aa, Homo sapiens
QSVLTQPPSVSGAPGQRVTISCTGSSSNIGAGYDVHWYQQLPGTAPKLLIYANSNRPSGVPDRFSGSKSGTSASLAITGLQAEDEANYYCQSYDSSLSVYVVFGGGTKLTVL

SEQ ID NO: 211 - protein, 126 aa, Homo sapiens
EVQLVQSGAELKKPGESLKISCKGSGFTFTNYWIAWVRQMPGKGLEWMGIIYPDDSDARYSPSFEGQVTISVDKSISTAYLQWSSLKASDTAIYYCARGGFCSGSVCYNPAWFDLWGQGTLVTVSS

SEQ ID NO: 212 - protein, 107 aa, Homo sapiens
DIQMTQSPSSLSASVGDRVTITCRASQTINTYLNWYLQKPGKAPKLLISDASSLETGVPSRFSGSGSGTDFTLTISSLQPDDFATYYCQQSYSTPLTFGGGTKVEIK

SEQ ID NO: 213 - protein, 121 aa, Homo sapiens
QVQLVQSGAEVKKPGASVKVSCKASGYTFTTHIIHWVRQAPGQRLEWMGWINAGNGNTHYSEKFQGRVTLTRDTSASTAYMELSSLRSEDTAIYYCAREDQWLGRSPLEYWGQGTLVTVSS

SEQ ID NO: 214 - protein, 109 aa, Homo sapiens
EIVLTQSPGTLSLSPGERATLSCRASQSVSSSYLAWYQHKPGQAPRLLIYGASSRATGIPDRFSGSGSGTDFTLTISRLEPEDFAVYYCQQYGNSYPWTFGQGTKVEIK

SEQ ID NO: 215 - protein, 121 aa, Homo sapiens
QVQLVQSGAEVKKPGASVKVSCKASGYTFTTHIIHWVRQAPGQRLEWMGWINAGNGNTKYSEKFQGRVTLTRDTSASTAYMELSSLRSEDTAIYYCAREDQWLGRSPLEYWGQGTLVTVSS

SEQ ID NO: 216 - protein, 109 aa, Homo sapiens
EIVLTQSPGTLSLSPGERATLSCRASQSVSSSYLAWYQHKPGQAPRLLIYGASSRATGIPDRFSGSGSGTDFTLTVSRLEPEDFAVYYCQQYGNSYPWTFGQGTKVEIK

SEQ ID NO: 217 - protein, 122 aa, Homo sapiens
EVQLSESGGGLVQPGGSLRLSCAASGFTFSSYAMSWVRQAPGKGLEWVSSLTGSGGSTYYRDSVKGRFTIFRDNSKKTLYMQMNSLRAEDTAVYYCAKEGAYSYDFWYFDLWGRGTLVTVSS

SEQ ID NO: 218 - protein, 107 aa, Homo sapiens
EIVLTQSPGTLSLSPGERATLSCRASQTVSGNYLAWYQQKPGQSPSLLIYGASSRATGIPDRFTGSGSGTDFTLTISRLEPADFAVYYCQQYGRPLTFGGGTKVDIK

SEQ ID NO: 219 - protein, 122 aa, Homo sapiens
EVQLLESGGGLVQPGGSLRLSCAASGFTFSSYAMSWVRQAPGKGLEWVSSLTGSGGSTYYRDSVKGRFTIFRDNSKKTLYMQMNSLRAEDTAVYYCAKEGAYSYDFWYFDLWGRGTLVTVSS

SEQ ID NO: 220 - protein, 107 aa, Homo sapiens
EIVLTQSPGTLSLSPGERATLSCRASQTVSGNYLAWYQQKPGQSPSLLTYGASSRATGIPDRFTGSGSGTDFTLTISRLEPADFAVYYCQQYGRPLTFGGGTKVEIK

SEQ ID NO: 221 - protein, 122 aa, Homo sapiens; identical to SEQ ID NO: 219

SEQ ID NO: 222 - protein, 107 aa, Homo sapiens
EIVLTQSPGTLSLSPGERATLSCRASQTVSGNYLAWYQQKPGQSPSLLIYGASSRATGIPDRFTGSGSGTDFTLTISRLEPADFAVYYCQQYGRPLTFGGGTKVEIK

SEQ ID NO: 223 - protein, 122 aa, Homo sapiens
EVQLLESGGGLVQPGGSLRLSCAASGFPFSSYAMSWVRQAPGKGLEWVSGITGSASGTYYADSVKGRFTISRDNSKNTLYLRMNSLRAEDTAVYYCAKEGAYSYDYWYFDLWGRGTLVTVSS

SEQ ID NO: 224 - protein, 107 aa, Homo sapiens
EIVLTQSPGTLSLSPGERATLSCRASQSVSGSYLAWYQQKPGQTPRLLIYGASSRATGIPDRFSGSGSGTDFTLTINRLDPEDFGVYYCQQYGSLVTFGGGSKVEIK

SEQ ID NO: 225 - protein, 126 aa, Homo sapiens
EVQLVESGGGVVQPGRSLRLSCAASGFTFSNFGMHWVRQPPGKGLEWVAVISYDGSDKFYADSVKGRFTISRDNFKNTLYVQMNSLRAEDTAVYYCAKDRVRTKYYYDHSGPFDYWGRGTLVTVSS

SEQ ID NO: 226 - protein, 108 aa, Homo sapiens
SYVLTQPPSVSVAPGQTARIACGGNNIGSKSVHWYQQRPGQAPVLVVYDDDDRPSGIPERFSGSNSGNTATLTISRVEAGDEADYFCQVWMTNSDRPVFGGGTKLTVL

SEQ ID NO: 227 - protein, 126 aa, Homo sapiens; identical to SEQ ID NO: 225

SEQ ID NO: 228 - protein, 108 aa, Homo sapiens
SYELTQPPSVSVAPGQTARIACGGNNIGSKSVHWYQQRPGQAPVLVVYDDDDRPSGIPERFSGSNSGNTATLTISRVEAGDEADYFCQVWMTNSDRPVFGGGTKLTVL

SEQ ID NO: 229 - protein, 126 aa, Homo sapiens
EVQLVESGGGVVQPGRSLRLSCAASGFTFSSYGMHWVRQAPGKGLEWVAVISKDGSNKYEADFVKGRFTISRDNSKNTLYLQMNSLRAEDTAVYYCAKIPLRRYSDSGDYSSGDFWGQGTLVTVSS

SEQ ID NO: 230 - protein, 113 aa, Homo sapiens
DVVMTQSPLSLTVTLGQPASISCRSSENLVYSDGNTYLSWFQQRPGQSPRRLIYKVSTRDSGVPDRFSGSGSGTDFTLKISRVEAEDVGVYYCMQTTHWPPLTFGGGTKVEIK

SEQ ID NO: 231 - protein, 120 aa, Homo sapiens
EVQLVESGGGVVQPGRSLRLSCAASGFIFNNHGMHWVRQAPGKGLEWVAGISYDGKKEYYIGSVKGRFTISRDNSRNTLYLHMNGLRPEDTAVYYCAKEAYGSGSPCDYWGQGTLVTVSS

SEQ ID NO: 232 - protein, 108 aa, Homo sapiens
EIVLTQSPGTLSLSPGERATLSCRASQRVSSNYLAWYQQKPGQAPRLLIYGASSRATGIPDRFSGSGSGTDFTLTISRLEPEDFAVYYCQQYGTSPRSFGRGTKLEIK

SEQ ID NO: 233 - protein, 119 aa, Homo sapiens
EVQLVESGGGLVQPGGSLRLSCAASGFSFGSYSMNWVRQAPGKGLEWVSHISSGSSSIYYADSVKGRFTISRDSVKNSLYLQMNNLRAEDTAVYYCARGWTGYDAFDIWGQGTMVTVSS

SEQ ID NO: 234 - protein, 107 aa, Homo sapiens
DIQMTQSPSSLSASVGDRVTITCRASQVISNYLAWYQEKPGKVPKLLIYAASTLQSGVPSRFSGSGTGTDFTLTIRSLQPEDVATYYCQKYNNAPLTFGGGTKVEIK

SEQ ID NO: 235 - protein, 119 aa, Homo sapiens
EVQLVESGGGLVHPGGSLRLSCAASGFRFGTYSMNWVRQAPGKGLEWVSHISSGSSSIYYADSVKGRFTISRDSVKNSLYLQMNNLRAEDTAVYFCARGWTGYDAFDIWGQGTMVTVSS

SEQ ID NO: 236 - protein, 107 aa, Homo sapiens
DIQMTQSPSSLSASVGDRVTITCRASQVISNYLAWYQEKPGEVPKLLIYAASTLQSGVPSRFSGSGTGTDFTLTISSLQPEDVATYYCQKYNNAPLTFGGGTKVEIK

SEQ ID NO: 237 - protein, 124 aa, Homo sapiens
EVQLVESGGGLVQPGGSLKLSCAASGFSLSNSEVHWVRQASGKGLEWIGRVRSRANRHATGYTESVNGRFTVSRDDSKNTASLQLESLKIEDTAVYYCTGVRGVISRYFAMDVWGQGTTVTVSS

SEQ ID NO: 238 - protein, 110 aa, Homo sapiens
QSALTQPASVSGSPGQSITISCTGTSSDVGAYNYVSWYRLRPGKDPHLIIYDVSHRPAGVSNRFSGSKSGNTASLTISGLQAEDEDEYYCCSYAHRGTPLFGGGTKLTVL

SEQ ID NO: 239 - protein, 124 aa, Homo sapiens
EVQLVQSGGGLVQPGGSLKLSCAASGFSSSGSEIHWVRQASGRGLEWIGRVRSTANRHAPGYTESVRGTFTVSRDESKNTASLELKSLKIEDTAVYYCTGVRGVISRYFAMDVWGQGTTVTVSS

SEQ ID NO: 240 - protein, 110 aa, Homo sapiens
QSALTQPASVSGSPGQSITISCTGTNSDLGSYNYVSWYRLHPGKDPHLIIYDVTHRPSGVSSRFSGSKSGKTASLTISGLQSEDEAEYFCCSYASVGSPIFGGGTKVTVL

SEQ ID NO: 241 - protein, 124 aa, Homo sapiens
EVQLVESGGGLVQPGGSLKLSCAASGFTFSGSEIHWVRQASGKGLEWIGRVRSRANRHATGYSESVKGRFTISRDDSKNTASLQLNSLKIEDTAVYYCTGVRGVISRYFAMDVWGQGTTVTVSS

SEQ ID NO: 242 - protein, 108 aa, Homo sapiens
SYVLTQTPSVSVAPGQTARITCGGNNIGSNSVHWYQQKPGQAPILVVYDDSERPSGIPERFSGSNSGNTATLTISRVEGGDEADYQCQVWDRRGDLLVFGGGTKLTVL

SEQ ID NO: 243 - protein, 129 aa, Homo sapiens
QLQLQESGPGLVQPSETLSLTCTVSGGYISTSSYYWGWIRQPPGKGLEWIGSIEYSGSTYYNPSLKSRVTISVDTSKNQFSLKLSSVTAADTAVYYCASANSKYYDSGGYYAPGALDLWGQGTMVTVSS

SEQ ID NO: 244 - protein, 109 aa, Homo sapiens
EIVMTQSPATLSVSPGERATLSCRASQSVSSHLAWYQHKRGQAPRLLIYAASSRATGIPARFSGRGSGTEFTLTISSLQSEDFAVYYCQQYNNWPPGYSFGQGTKLEIK

SEQ ID NO: 245 - protein, 129 aa, Homo sapiens
QLQLQESGPGLVKPSETLSLTCTVSGTYISTNSYYWGWIRQPPGKGLEWIGSIEYGGSTYYNPSLRSRLTISVDTSKNHFSLRLSSVTAADTAMYYCASANSHYYDSGGYCAPSALDIWGQGTMVTVSS

SEQ ID NO: 246 - protein, 109 aa, Homo sapiens
EIVMTQSPATLSVSPGERVTLSCRASQSASSHLAWYQHKRGQAPRLLIYAASSRATGIPARFSGRGSGTEFTLTISSLQSEDFAVYYCQQYNNWPPGYSFGQGTKLEIK

SEQ ID NO: 247 - protein, 121 aa, Homo sapiens
QVQLQESGPGLVKPSQTLSLTCSVSGGSISSGNYYWSWIRQPAGKGLEWIGRIYTSGNTNYNPSLKSRVTMSVDTSKNQFSLKLSSVTATDTAVYYCARVRRDGYNAFDYWGQGTLVTVSS

SEQ ID NO: 248 - protein, 107 aa, Homo sapiens
SYELTQPPSVSVSPGQTASIDCSGHNLGDKFTCWYQQKPGQSPVLVIYQDSKRPSGIPERFSGSNSGNTATLTISGTQAMDEADYYCQAWDSDTLYVFGTGTTVTVL

SEQ ID NO: 249 - protein, 123 aa, Homo sapiens
QVQLQESGPGLVRPSQTLSLTCTVSGGSMTSGSYYWSWIRQPAEKGLEWIGRIYTSGRTDYNPSLKSRVAMSIDTSKNQFSLRLTSVTAADTAVYYCARWGDSSAYYYVGDPWGRGTTVTVSS

SEQ ID NO: 250 - protein, 107 aa, Homo sapiens
DIQMTQSPSSLSASIGDRVTITCRASQNINTYLYWYQQKPGKAPQLLIYAASNLQTGAPSRFSGSGSGTDFTLTISSLQPADFATYYCQQSFSLPHTFGQGTKLEIK

SEQ ID NO: 251 - protein, 123 aa, Homo sapiens
QVQLQESGPGLVRPSQTLSLTCTVSGGSMTSGSYYWSWIRQPAEKGLEWIGRIYTSGRTDYNPSLKSRVAMSIDTSKNQFSLRLTSVTAADTAVYYCARWGDSSAYYYVGDPWGRGTPVTVSS

SEQ ID NO: 252 - protein, 107 aa, Homo sapiens
DIQMTQSPSSLSASIGDRVTITCRASQNINTYLYWYQQKPGKAPQLLIYAASNLQTGAPSRFSGSGSGTDFTLTISSLQPADFATYYCQQSFSLPHTFGQGTKVEIK

SEQ ID NO: 253 - protein, 123 aa, Homo sapiens; identical to SEQ ID NO: 251

SEQ ID NO: 254 - protein, 107 aa, Homo sapiens; identical to SEQ ID NO: 250

SEQ ID NO: 255 - protein, 130 aa, Homo sapiens
QVQLVQSGSEVKKPGTSVKVSCKASGETYVGHSISWVRQAPGAGLEWMGWISLHNGNVKYAQKLQGRVTMTTDTSTITAYMELRNLTSDDTAVYYCARVPMKIYGVIVFGEYYYDQLDVWGQGTTVTVSS

SEQ ID NO: 256 - protein, 109 aa, Homo sapiens
QSALTQPPSASGSPGQSVTISCTGTGSDVGGYNYVSWYQQHPGKAPKLMIYEVSKRPSGVPDRFSGSKSGNTASLTVSGLQAEDEADYYCSSYAGSKVVFGGGTKLTVL

SEQ ID NO: 257 - protein, 126 aa, Homo sapiens
QVQLVQSGAEVKKPGASVKVSCKVSGYTFTSYSMHWLRQAPGQRLEWMGWINAGNGDTKYSQKFQGRITISRDTSARTTYMELSSLRSEDTAVFYCARSNSPTVTYNYYYYAMDVWGQGTTVTVSS

SEQ ID NO: 258 - protein, 108 aa, Homo sapiens
EIVLTQSPGTLSLSPGERATLSCRASQSVRSSYLAWYQQQAGQAPRLLIYDASSRATGIPDRFSGSGSGTDFSLTISRLDPEDFAVYYCQQYGNSPLTFGGGTKVEIK

SEQ ID NO: 259 - protein, 124 aa, Homo sapiens
QVQLVQSGAEVKKPGSSVKVSCKASGGRFSRYGSSWVRQAPGQGLEWMGGIIPLLGTANYAQKFQDRVSITADESTSTVYMHLSSLRSEDTAVYYCATARREYDRPGAEYFIQWGQGTLVTVSS

SEQ ID NO: 260 - protein, 108 aa, Homo sapiens
EIVMTQSPATLSVSPGERATLSCRASQSVSTNLAWYQQKPGQAPRLLIYDAFLRATGIPARFSGSGSGTEFTLTISSLQPEDFAVYYCQQYNYWPPLTFGGGTKVEIK

SEQ ID NO: 261 - protein, 122 aa, Homo sapiens; identical to SEQ ID NO: 177

SEQ ID NO: 262 - protein, 110 aa, Homo sapiens; identical to SEQ ID NO: 238

SEQ ID NO: 263 - protein, 123 aa, Homo sapiens
EVQLLESGGALVQPGGSLRLSCAASGFTFRSYAMNWVRQAPGKGLEWVSSLSSSGTTTYYADSVKGRFTISRDNSKNTMYLQMDSLRGEDTAVYYCAKDRNAQWLGSEPLDPWGQGTLVTVSS

SEQ ID NO: 264 - protein, 108 aa, Homo sapiens
EIVLTQSPGTLSLSPGERATLSCRASQSVSSSYLAWYQQKPGQAPRLLIYGASSRATGIPDRFSGSGSGTDFTLTISSLQPDDFAIYYCQQAYTFPWTFGQGTKLEIK

SEQ ID NO: 265 - protein, 117 aa, Homo sapiens
EVQLLESGGGLVQPGGSLRLSCVTSGFTFSSYSMTWVRQAPGKGLEWVSYISSSSRTISYADSVQGRFTISRDNAKNVLYLQMNSLRAEDTAVYYCARQAVAHFDYWGQGTLVTVSS

SEQ ID NO: 266 - protein, 108 aa, Homo sapiens
EIVLTQSPGTLSLSPGERATLSCRASQRVSSNYLAWYQQKPGQAPRLLIYGASSRATGIPDRFSGSGSGTDFTLTISRLEPEDFAVYYCQQYGTSPRSFGQGTKVEIK

SEQ ID NO: 267 - protein, 121 aa, Homo sapiens
EVQLVESGGGLVQPGGSLRLSCSASGFTFSTYTMNWVRQAPGKGLDWVSYISSRSTSIYYADSVKGRFTISRDNAKNSLYLHMTSLRAEDTAVYYCVRDRGYYGSNWFDSWGQGTLVTVSS

SEQ ID NO: 268 - protein, 110 aa, Homo sapiens
QSALTQPRSVSGSPGQSVTISCTGTSSDVGNYNYVSWYQQHPGKAPRLMISDVTKRPSGVPDRFSGSKSGNTASLTISGLQAEDEGDYYCCAYAGSYTLVFGGGTKLTVL

SEQ ID NO: 269 - protein, 123 aa, Homo sapiens
QVQLQESGPGLVKPSQTLSLTCTVSGGSISSGRYYWSWIRQPAGKGLEWIGRVYFSGSTNYNPSLKNRVTLSVDTSKNQFSLKLSSVIAADTAVYYCARAVRDYGDSYSFDYWGQGTLVTVSS

SEQ ID NO: 270 - protein, 110 aa, Homo sapiens
QSALTQPASVSGSPGQSITISCTGSSSDIGGYNYVSWYQVHPGKAPHLKIYDVVNRPSGVSNRFPGSKSGNTASLTISGLLADDEAYYYCCSYSIRGTPVFGGGTKLTVL

SEQ ID NO: 271 - protein, 362 aa, Homo sapiens
MAPTKRKGECPGAAPKKPKEPVQVPKLLIKGGVEVLEVKTGVDAITEVECFLNPEMGDPDENLRGFSLKLSAENDFSSDSPERKMLPCYSTARIPLPNLNEDLTCGNLLMWEAVTVQTEVIGITSMLNLHAGSQKVHEHGGGKPIQGSNFHFFAVGGEPLEMQGVLMNYRSKYPDGTITPKNPTAQSQVMNTDHKAYLDKNNAYPVECWVPDPSRNENARYFGTFTGGENVPPVLHVTNTATTVLLDEQGVGPLCKADSLYVSAADICGLFTNSSGTQQWRGLARYFKIRLRKRSVKNPYPISFLLSDLINRRTQRVDGQPMYGMESQVEEVRVFDGTERLPGDPDMIRYIDKQGQLQTKML

SEQ ID NO: 272 - protein, 362 aa, Homo sapiens
MAPTKRKGECPGAAPKKPKEPVQVPKLLIKGGVEVLEVKTGVDAITEVECFLNPEMGDPDDNLRGYSLKLTAENAFDSDSPDKKMLPCYSTARIPLPNLNEDLTCGNLLMWEAVTVKTEVIGITSMLNLHAGSQKVHENGGGKPVQGSNFHFFAVGGDPLEMQGVLMNYRTKYPQGTITPKNPTAQSQVMNTDHKAYLDKNNAYPVECWIPDPSRNENTRYFGTYTGGENVPPVLHVTNTATTVLLDEQGVGPLCKADSLYVSAADICGLFTNSSGTQQWRGLARYFKIRLRKRSVKNPYPISFLLSDLINRRTQKVDGQPMYGMESQVEEVRVFDGTEQLPGDPDMIRYIDRQGQLQTKMV

SEQ ID NO: 273 - protein, 362 aa, Homo sapiens
MAPTKRKGECPGAAPKKPKEPVQVPKLLIKGGVEVLEVKTGVDAITEVECFLNPEMGDPDNDLRGYSLRLTAETAFDSDSPDRKMLPCYSTARIPLPNLNEDLTCGNLLMWEAVTVKTEVIGITSMLNLHAGSQKVHENGGGKPIQGSNFHFFAVGGDPLEMQGVLMNYRTKYPEGTVTPKNPTAQSQVMNTDHKAYLDKNNAYPVECWIPDPSRNENTRYFGTYTGGENVPPVLHVTNTATTVLLDEQGVGPLCKADSLYVSAADICGLFTNSSGTQQWRGLPRYFKIRLRKRSVKNPYPISFLLSDLINRRTQRVDGQPMYGMESQVEEVRVFDGTEQLPGDPDMIRYIDRQGQLQTKMV

SEQ ID NO: 274 - protein, 354 aa, Homo sapiens
MAPTKRKGERKDPVQVPKLLIRGGVEVLEVKTGVDSITEVECFLTPEMGDPDEHLRGFSKSISISDTFESDSPNRDMLPCYSVARIPLPNLNEDLTCGNILMWEAVTLKTEVIGVTSLMNVHSNGQATHDNGAGKPVQGTSFHFFSVGGEALELQGVLFNYRTKYPDGTIFPKNATVQSQVMNTEHKAYLDKNKAYPVECWVPDPTRNENTRYFGTLTGGENVPPVLHITNTATTVLLDEFGVGPLCKGDNLYLSAVDVCGMFTNRSGSQQWRGLSRYFKVQLRKRRVKNPYPISFLLTDLINRRTPRVDGQPMYGMDAQVEEVRVFEGTEELPGDPDMMRYVDKYGQLQTKML